European Patent Application EP 4 786 497 A1, published August 5, 2026. Title: Anti-MerTK agonist antibody, anti-MerTK bispecific antibody and uses thereof. Applicant: Astellas Pharma Inc. The sequence listing filed with the application follows.

SEQUENCE LISTING (70 sequences)

SEQ ID NO: 1 - protein, 5 aa, synthetic construct
  source 1..5: note = tA3-20_tA3-20.5_HC_CDR1_aa
SYAIS

SEQ ID NO: 2 - protein, 17 aa, synthetic construct
  source 1..17: note = tA3-20_tA3-20.5_HC_CDR2_aa
GIIPIFGPAKHAQKFQG

SEQ ID NO: 3 - protein, 10 aa, synthetic construct
  source 1..10: note = tA3-20_tA3-20.5_HC_CDR3_aa
LVGATGWFDP

SEQ ID NO: 4 - protein, 13 aa, synthetic construct
  source 1..13: note = tA3-20_tA3-20.5_LC_CDR1_aa
TRSSGSIATNYVQ

SEQ ID NO: 5 - protein, 7 aa, synthetic construct
  source 1..7: note = tA3-20_tA3-20.5_LC_CDR2_aa
EDNQRPS

SEQ ID NO: 6 - protein, 9 aa, synthetic construct
  source 1..9: note = tA3-20_tA3-20.5_LC_CDR3_aa
QSYDSSNVV

SEQ ID NO: 7 - DNA, 1347 bp, synthetic construct
  source 1..1347: mol_type = other DNA; note = tA3-20_tA3-20.5_HC_DNA
caggtgcagctggttcagtctggcgccgaagtgaagaaacctggctcctccgtgaaggtgtcctgcaaggcttctggcggcaccttcaactcctacgccatctcttggatgagacaggcccctggacagggccttgaatggatgggaggcatcatccccatcttcggccctgctaagcacgcccagaaattccagggcagagtgaccatcaccgccgacaagtctacctccaccgtgtacatggaactgtccagcctgagatccgaggacaccgccgtgtactactgtgctagactcgtgggcgctaccggatggttcgatccttggggacagggcacactggtcaccgtgtcctctgcttctaccaagggacccagcgtgttccctctggctcctagctctaagtccacctccggtggaacagctgctctgggctgtctggtcaaggactacttccctgagcctgtgaccgtgtcttggaactctggcgctctgacatccggcgtgcacacctttccagctgtgctgcaatcctccggcctgtactctctgtcctccgtcgtgaccgtgccttctagctctctgggcacccagacctacatctgcaatgtgaaccacaagccttccaacaccaaggtggacaagaaggtggaacccaagtcctgcgacaagacccacacctgtcctccatgtcctgctccagaagctgcaggcggcccttccgtgtttctgttccctccaaagcctaaggacaccctgatgatctctcggacccctgaagtgacctgcgtggtggtggatgtgtctcacgaggacccagaagtgaagttcaattggtacgtggacggcgtggaagtgcacaacgccaagaccaagcctagagaggaacagtacaactccacctacagagtggtgtccgtgctgaccgtgctgcaccaggattggctgaacggcaaagagtacaagtgcaaggtgtccaacaaggcactgcctgccggcatcgaaaagaccatctccaaggctaagggccagcctcgggaaccccaggtttacacattgcctccatctcgggacgagctgaccaagaaccaggtgtccctgacctgtctcgtgaagggcttctacccctccgatatcgccgtggaatgggagtccaatggccagccagagaacaactacaagacaacccctcctgtgctggactccgacggctcattcttcctgtactccaagctgacagtggacaagtccagatggcagcagggcaacgtgttctcctgctccgtgatgcacgaggccctgcacaatcactacacacagaagtccctgtctctgtcccctggcaag

SEQ ID NO: 8 - protein, 449 aa, synthetic construct
  source 1..449: note = tA3-20_tA3-20.5_HC_aa
QVQLVQSGAEVKKPGSSVKVSCKASGGTFNSYAISWMRQAPGQGLEWMGGIIPIFGPAKHAQKFQGRVTITADKSTSTVYMELSSLRSEDTAVYYCARLVGATGWFDPWGQGTLVTVSSASTKGPSVFPLAPSSKSTSGGTAALGCLVKDYFPEPVTVSWNSGALTSGVHTFPAVLQSSGLYSLSSVVTVPSSSLGTQTYICNVNHKPSNTKVDKKVEPKSCDKTHTCPPCPAPEAAGGPSVFLFPPKPKDTLMISRTPEVTCVVVDVSHEDPEVKFNWYVDGVEVHNAKTKPREEQYNSTYRVVSVLTVLHQDWLNGKEYKCKVSNKALPAGIEKTISKAKGQPREPQVYTLPPSRDELTKNQVSLTCLVKGFYPSDIAVEWESNGQPENNYKTTPPVLDSDGSFFLYSKLTVDKSRWQQGNVFSCSVMHEALHNHYTQKSLSLSPGK

SEQ ID NO: 9 - DNA, 645 bp, synthetic construct
  source 1..645: mol_type = other DNA; note = tA3-20_LC_DNA
ttcatgctgacccagcctcactccgtgtctgagtctccaggcaagaccgtgaacatcagctgcaccagatcctccggctctatcgccaccaactacgtgcagtggtatcagcagaggcccggctcctctcctaccaccgtgatctacgaggacaaccagaggccttctggcgtgcccgatagattttccggctccatcgactcctccagcaactccgcttctctgaccatctccggcctgaaaaccgaggacgaggccgtgtaccactgccagtcctacgactcctctaacgtggtgtttggcggaggcaccaagctgacagtgctgggacaacctaaggccgctccttccgtgacactgttccctccatcctccgaggaactgcaggccaacaaggctaccctcgtgtgcctgatctccgacttttaccctggcgctgtgaccgtggcctggaaggctgatagttctcctgtgaaggccggcgtggaaaccaccacaccttccaagcagtccaacaacaaatacgccgcctcctcctacctgtctctgacccctgaacagtggaagtcccaccggtcctacagctgccaagtgacccatgagggctccaccgtggaaaagaccgtggctcctaccgagtgctcc

SEQ ID NO: 10 - protein, 215 aa, synthetic construct
  source 1..215: note = tA3-20_LC_aa
FMLTQPHSVSESPGKTVNISCTRSSGSIATNYVQWYQQRPGSSPTTVIYEDNQRPSGVPDRFSGSIDSSSNSASLTISGLKTEDEAVYHCQSYDSSNVVFGGGTKLTVLGQPKAAPSVTLFPPSSEELQANKATLVCLISDFYPGAVTVAWKADSSPVKAGVETTTPSKQSNNKYAASSYLSLTPEQWKSHRSYSCQVTHEGSTVEKTVAPTECS

SEQ ID NO: 11 - DNA, 645 bp, synthetic construct
  source 1..645: mol_type = other DNA; note = tA3-20.1_LC_DNA
ttcatgctgacccagcctcactccgtgtctgagtctccaggcaagaccgtgaccatcagctgcaccagatcctccggctctatcgccaccaactacgtgcagtggtatcagcagaggcccggctcctctcctaccaccgtgatctacgaggacaaccagaggccttctggcgtgcccgatagattttccggctccatcgactcctccagcaactccgcttctctgaccatctccggcctgaaaaccgaggacgaggccgtgtaccactgccagtcctacgactcctctaacgtggtgtttggcggaggcaccaagctgacagtgctgggacaacctaaggccgctccttccgtgacactgttccctccatcctccgaggaactgcaggccaacaaggctaccctcgtgtgcctgatctccgacttttaccctggcgctgtgaccgtggcctggaaggctgatagttctcctgtgaaggccggcgtggaaaccaccacaccttccaagcagtccaacaacaaatacgccgcctcctcctacctgtctctgacccctgaacagtggaagtcccaccggtcctacagctgccaagtgacccatgagggctccaccgtggaaaagaccgtggctcctaccgagtgctcc

SEQ ID NO: 12 - protein, 215 aa, synthetic construct
  source 1..215: note = tA3-20.1_LC_aa
FMLTQPHSVSESPGKTVTISCTRSSGSIATNYVQWYQQRPGSSPTTVIYEDNQRPSGVPDRFSGSIDSSSNSASLTISGLKTEDEAVYHCQSYDSSNVVFGGGTKLTVLGQPKAAPSVTLFPPSSEELQANKATLVCLISDFYPGAVTVAWKADSSPVKAGVETTTPSKQSNNKYAASSYLSLTPEQWKSHRSYSCQVTHEGSTVEKTVAPTECS

SEQ ID NO: 13 - DNA, 645 bp, synthetic construct
  source 1..645: mol_type = other DNA; note = tA3-20.2_LC_DNA
ttcatgctgacccagcctcactccgtgtctgagtctccaggcaagaccgtgagcatcagctgcaccagatcctccggctctatcgccaccaactacgtgcagtggtatcagcagaggcccggctcctctcctaccaccgtgatctacgaggacaaccagaggccttctggcgtgcccgatagattttccggctccatcgactcctccagcaactccgcttctctgaccatctccggcctgaaaaccgaggacgaggccgtgtaccactgccagtcctacgactcctctaacgtggtgtttggcggaggcaccaagctgacagtgctgggacaacctaaggccgctccttccgtgacactgttccctccatcctccgaggaactgcaggccaacaaggctaccctcgtgtgcctgatctccgacttttaccctggcgctgtgaccgtggcctggaaggctgatagttctcctgtgaaggccggcgtggaaaccaccacaccttccaagcagtccaacaacaaatacgccgcctcctcctacctgtctctgacccctgaacagtggaagtcccaccggtcctacagctgccaagtgacccatgagggctccaccgtggaaaagaccgtggctcctaccgagtgctcc

SEQ ID NO: 14 - protein, 215 aa, synthetic construct
  source 1..215: note = tA3-20.2_LC_aa
FMLTQPHSVSESPGKTVSISCTRSSGSIATNYVQWYQQRPGSSPTTVIYEDNQRPSGVPDRFSGSIDSSSNSASLTISGLKTEDEAVYHCQSYDSSNVVFGGGTKLTVLGQPKAAPSVTLFPPSSEELQANKATLVCLISDFYPGAVTVAWKADSSPVKAGVETTTPSKQSNNKYAASSYLSLTPEQWKSHRSYSCQVTHEGSTVEKTVAPTECS

SEQ ID NO: 15 - DNA, 648 bp, synthetic construct
  source 1..648: mol_type = other DNA; note = tA3-20.3_LC_DNA
aacttcatgctgacccagcctcactccgtgtctgagtctccaggcaagaccgtgaacatcagctgcaccagatcctccggctctatcgccaccaactacgtgcagtggtatcagcagaggcccggctcctctcctaccaccgtgatctacgaggacaaccagaggccttctggcgtgcccgatagattttccggctccatcgactcctccagcaactccgcttctctgaccatctccggcctgaaaaccgaggacgaggccgtgtaccactgccagtcctacgactcctctaacgtggtgtttggcggaggcaccaagctgacagtgctgggacaacctaaggccgctccttccgtgacactgttccctccatcctccgaggaactgcaggccaacaaggctaccctcgtgtgcctgatctccgacttttaccctggcgctgtgaccgtggcctggaaggctgatagttctcctgtgaaggccggcgtggaaaccaccacaccttccaagcagtccaacaacaaatacgccgcctcctcctacctgtctctgacccctgaacagtggaagtcccaccggtcctacagctgccaagtgacccatgagggctccaccgtggaaaagaccgtggctcctaccgagtgctcc

SEQ ID NO: 16 - protein, 216 aa, synthetic construct
  source 1..216: note = tA3-20.3_LC_aa
NFMLTQPHSVSESPGKTVNISCTRSSGSIATNYVQWYQQRPGSSPTTVIYEDNQRPSGVPDRFSGSIDSSSNSASLTISGLKTEDEAVYHCQSYDSSNVVFGGGTKLTVLGQPKAAPSVTLFPPSSEELQANKATLVCLISDFYPGAVTVAWKADSSPVKAGVETTTPSKQSNNKYAASSYLSLTPEQWKSHRSYSCQVTHEGSTVEKTVAPTECS

SEQ ID NO: 17 - DNA, 648 bp, synthetic construct
  source 1..648: mol_type = other DNA; note = tA3-20.4_LC_DNA
aacttcatgctgacccagcctcactccgtgtctgagtctccaggcaagaccgtgaccatcagctgcaccagatcctccggctctatcgccaccaactacgtgcagtggtatcagcagaggcccggctcctctcctaccaccgtgatctacgaggacaaccagaggccttctggcgtgcccgatagattttccggctccatcgactcctccagcaactccgcttctctgaccatctccggcctgaaaaccgaggacgaggccgtgtaccactgccagtcctacgactcctctaacgtggtgtttggcggaggcaccaagctgacagtgctgggacaacctaaggccgctccttccgtgacactgttccctccatcctccgaggaactgcaggccaacaaggctaccctcgtgtgcctgatctccgacttttaccctggcgctgtgaccgtggcctggaaggctgatagttctcctgtgaaggccggcgtggaaaccaccacaccttccaagcagtccaacaacaaatacgccgcctcctcctacctgtctctgacccctgaacagtggaagtcccaccggtcctacagctgccaagtgacccatgagggctccaccgtggaaaagaccgtggctcctaccgagtgctcc

SEQ ID NO: 18 - protein, 216 aa, synthetic construct
  source 1..216: note = tA3-20.4_LC_aa
NFMLTQPHSVSESPGKTVTISCTRSSGSIATNYVQWYQQRPGSSPTTVIYEDNQRPSGVPDRFSGSIDSSSNSASLTISGLKTEDEAVYHCQSYDSSNVVFGGGTKLTVLGQPKAAPSVTLFPPSSEELQANKATLVCLISDFYPGAVTVAWKADSSPVKAGVETTTPSKQSNNKYAASSYLSLTPEQWKSHRSYSCQVTHEGSTVEKTVAPTECS

SEQ ID NO: 19 - DNA, 648 bp, synthetic construct
  source 1..648: mol_type = other DNA; note = tA3-20.5_LC_DNA
aacttcatgctgacccagcctcactccgtgtctgagtctccaggcaagaccgtgagcatcagctgcaccagatcctccggctctatcgccaccaactacgtgcagtggtatcagcagaggcccggctcctctcctaccaccgtgatctacgaggacaaccagaggccttctggcgtgcccgatagattttccggctccatcgactcctccagcaactccgcttctctgaccatctccggcctgaaaaccgaggacgaggccgtgtaccactgccagtcctacgactcctctaacgtggtgtttggcggaggcaccaagctgacagtgctgggacaacctaaggccgctccttccgtgacactgttccctccatcctccgaggaactgcaggccaacaaggctaccctcgtgtgcctgatctccgacttttaccctggcgctgtgaccgtggcctggaaggctgatagttctcctgtgaaggccggcgtggaaaccaccacaccttccaagcagtccaacaacaaatacgccgcctcctcctacctgtctctgacccctgaacagtggaagtcccaccggtcctacagctgccaagtgacccatgagggctccaccgtggaaaagaccgtggctcctaccgagtgctcc

SEQ ID NO: 20 - protein, 216 aa, synthetic construct
  source 1..216: note = tA3-20.5_LC_aa
NFMLTQPHSVSESPGKTVSISCTRSSGSIATNYVQWYQQRPGSSPTTVIYEDNQRPSGVPDRFSGSIDSSSNSASLTISGLKTEDEAVYHCQSYDSSNVVFGGGTKLTVLGQPKAAPSVTLFPPSSEELQANKATLVCLISDFYPGAVTVAWKADSSPVKAGVETTTPSKQSNNKYAASSYLSLTPEQWKSHRSYSCQVTHEGSTVEKTVAPTECS

SEQ ID NO: 21 - DNA, 18 bp, synthetic construct
  source 1..18: mol_type = other DNA; note = Histag_DNA
catcatcatcatcatcac

SEQ ID NO: 22 - protein, 6 aa, synthetic construct
  source 1..6: note = Histag_aa
HHHHHH

SEQ ID NO: 23 - DNA, 1344 bp, synthetic construct
  source 1..1344: mol_type = other DNA; note = MTK201_HC_DNA
caggtccagctgagacagtctggccctggactggttcagccttctcagtccctgtccatcacctgtaccgtgtccggcttctccctgtctaactacggcctgcactgggtccgacagtctccaggcaaaggactggaatggctgggagtgatttggagcggcggcatcaccgattacaacgccgccttcatctcccggctgagcatcatcaaggacaactctcggagccaggtgttcttcaagatgaactccctgcaggccgacgacaccgccatctactactgtgccagaaagggccacgatccttacgccatggatttctggggccagggcacctctgtgaccgtgtctagcgcttctaccaagggacccagcgtgttccctctggctccttccagcaagtctacctctggcggaacagctgctctgggctgcctggtcaaggactactttcctgagcctgtgacagtgtcctggaactctggcgctctgacatccggcgtgcacacctttccagctgtgctgcaatcctccggcctgtactctctgtcctccgtcgtgaccgtgccttctagctctctgggcacccagacctacatctgcaatgtgaaccacaagccttccaacaccaaggtggacaagaaggtggaacccaagtcctgcgacaagacccacacctgtcctccatgtcctgctccagaagctgctggcggcccttccgtgtttctgttccctccaaagcctaaggacaccctgatgatctctcggacccctgaagtgacctgcgtggtggtggatgtgtctcacgaggatcccgaagtgaagttcaattggtacgtggacggcgtggaagtgcacaacgccaagaccaagcctagagaggaacagtacaactccacctacagagtggtgtccgtgctgaccgtgctgcaccaggattggctgaacggcaaagagtacaagtgcaaggtgtccaacaaggccctgcctgccggcatcgaaaagaccatctctaaggccaagggccagcctcgggaaccccaggtttacacattgcctccatctcgggacgagctgaccaagaaccaggtgtccctgacctgtctcgtgaagggcttctacccctccgatatcgccgtggaatgggagtctaatggccagcctgagaacaactacaagacaacccctcctgtgctggactccgacggctcattcttcctgtactccaagctgacagtggacaagtccagatggcagcagggcaacgtgttctcctgctccgtgatgcacgaggccctgcacaatcactacacccagaagtctctgtctctgtcccctggcaag

SEQ ID NO: 24 - protein, 448 aa, synthetic construct
  source 1..448: note = MTK201_HC_aa
QVQLRQSGPGLVQPSQSLSITCTVSGFSLSNYGLHWVRQSPGKGLEWLGVIWSGGITDYNAAFISRLSIIKDNSRSQVFFKMNSLQADDTAIYYCARKGHDPYAMDFWGQGTSVTVSSASTKGPSVFPLAPSSKSTSGGTAALGCLVKDYFPEPVTVSWNSGALTSGVHTFPAVLQSSGLYSLSSVVTVPSSSLGTQTYICNVNHKPSNTKVDKKVEPKSCDKTHTCPPCPAPEAAGGPSVFLFPPKPKDTLMISRTPEVTCVVVDVSHEDPEVKFNWYVDGVEVHNAKTKPREEQYNSTYRVVSVLTVLHQDWLNGKEYKCKVSNKALPAGIEKTISKAKGQPREPQVYTLPPSRDELTKNQVSLTCLVKGFYPSDIAVEWESNGQPENNYKTTPPVLDSDGSFFLYSKLTVDKSRWQQGNVFSCSVMHEALHNHYTQKSLSLSPGK

SEQ ID NO: 25 - DNA, 645 bp, synthetic construct
  source 1..645: mol_type = other DNA; note = MTK201_LC_DNA
cagatcgtgctgacccagtctcctcctatcatgtccgcctttctcggcgagcgcgtgacaatgacctgtaccgcctcttccagcgtgtcctcctcttacctgcactggtacagacagatgcccggcagctctcccaagctgtggatctacgacacctccaacctggcctctggcgtgccagctagattttccggctctggctctggcacctcctacagcctgaccatctcctccatggaagccgaggatgccgccacctactactgccaccagtaccaccactctccatacacctttggcggaggcaccaagctggaaatcaagcggacagtggccgctccttccgtgttcatcttcccaccttccgacgagcagctgaagtctggcacagcctctgtcgtgtgcctgctgaacaacttctaccctcgggaagccaaggtgcagtggaaggtggacaatgccctgcagtccggcaactcccaagagtctgtgaccgagcaggactccaaggactctacctactctctgtcctccacactgaccctgtccaaggccgactacgagaagcacaaggtgtacgcctgcgaagtgacccatcagggcctgtctagccctgtgaccaagtctttcaaccggggcgagtgc

SEQ ID NO: 26 - protein, 215 aa, synthetic construct
  source 1..215: note = MTK201_LC_aa
QIVLTQSPPIMSAFLGERVTMTCTASSSVSSSYLHWYRQMPGSSPKLWIYDTSNLASGVPARFSGSGSGTSYSLTISSMEAEDAATYYCHQYHHSPYTFGGGTKLEIKRTVAAPSVFIFPPSDEQLKSGTASVVCLLNNFYPREAKVQWKVDNALQSGNSQESVTEQDSKDSTYSLSSTLTLSKADYEKHKVYACEVTHQGLSSPVTKSFNRGEC

SEQ ID NO: 27 - protein, 5 aa, synthetic construct
  source 1..5: note = 371M_HC_CDR1_aa
SYAMS

SEQ ID NO: 28 - protein, 17 aa, synthetic construct
  source 1..17: note = 371M_HC_CDR2_aa
AISGSGGSTYYADSVKG

SEQ ID NO: 29 - protein, 10 aa, synthetic construct
  source 1..10: note = 371M_HC_CDR3_aa
GTRTNWYFDL

SEQ ID NO: 30 - protein, 15 aa, synthetic construct
  source 1..15: note = 371M_LC_CDR1_aa
SCSGSRSNIGSNTVN

SEQ ID NO: 31 - protein, 7 aa, synthetic construct
  source 1..7: note = 371M_LC_CDR2_aa
SNNQRPS

SEQ ID NO: 32 - protein, 11 aa, synthetic construct
  source 1..11: note = 371M_LC_CDR3_aa
AAWDDSLYGPV

SEQ ID NO: 33 - DNA, 1347 bp, synthetic construct
  source 1..1347: mol_type = other DNA; note = tA3-20.3_mouse_HC
caggtgcagctggtgcagtctggggctgaggtgaagaagcctgggtcctcggtgaaggtctcctgcaaggcttctggaggcaccttcaacagctatgctatcagctggatgcgacaggcccctggacaaggacttgagtggatgggagggatcatccctatctttggtccagcaaaacacgcacagaagttccagggcagagtcacgattaccgcggacaaatccacgagcacagtgtacatggagttgagcagcctgagatctgaggacacggccgtgtattattgtgcgagactagtgggagctactggctggttcgacccctggggccagggaaccctggtcaccgtctcctcagctaagaccaccgctcctagcgtgtaccctctggctcctgtgtgtggcgataccaccggatcttccgtgacactgggctgtctggtcaagggctacttccccgaacctgtgacactgacctggaactccggctctctgtctagcggcgtgcacacctttccagccgtgctgcagtctgacctgtacaccctgtcctctagcgtgaccgtgacctcctctacctggcctagccagtccatcacctgtaacgtggcccatcctgcctccagcaccaaggtggacaagaagatcgagcctcggggccctaccatcaagccttgtcctccatgcaagtgccccgctcctaatgctgctggtggcccttccgtgttcatcttcccacctaagatcaaggacgtgctgatgatctccctgtctcctatcgtgacctgcgtggtggtggacgtgtccgaggatgatcctgacgtgcagatcagttggttcgtgaacaacgtggaagtgcacaccgctcagacccagacacacagagaggactacaacagcaccctgagagtggtgtctgccctgcctatccagcatcaggactggatgtccggcaaagagttcaagtgcaaagtgaacaacaaggacctggccgctcctatcgagcggaccatctctaagcctaagggctctgtcagggcccctcaggtgtacgttttgccacctcctgagaaagagatgaccaagaaacaggtgtccctgacctgcctcgtgaaggacttcatgcccgaggacatctacgtggaatggaccaacaacggcaagaccgagctgaactacaagaacaccgagcctgtgctgaagtccgacggctcctacttcatgtactccaagctgaccgtcgagaagaagaactgggtcgagagaaactcctactcctgctccgtggtgcacgagggcctgcacaatcaccacaccaccaagtccttctctcggacccctggaaag

SEQ ID NO: 34 - protein, 449 aa, synthetic construct
  source 1..449: note = tA3-20.3_mouse_HC
QVQLVQSGAEVKKPGSSVKVSCKASGGTFNSYAISWMRQAPGQGLEWMGGIIPIFGPAKHAQKFQGRVTITADKSTSTVYMELSSLRSEDTAVYYCARLVGATGWFDPWGQGTLVTVSSAKTTAPSVYPLAPVCGDTTGSSVTLGCLVKGYFPEPVTLTWNSGSLSSGVHTFPAVLQSDLYTLSSSVTVTSSTWPSQSITCNVAHPASSTKVDKKIEPRGPTIKPCPPCKCPAPNAAGGPSVFIFPPKIKDVLMISLSPIVTCVVVDVSEDDPDVQISWFVNNVEVHTAQTQTHREDYNSTLRVVSALPIQHQDWMSGKEFKCKVNNKDLAAPIERTISKPKGSVRAPQVYVLPPPEKEMTKKQVSLTCLVKDFMPEDIYVEWTNNGKTELNYKNTEPVLKSDGSYFMYSKLTVEKKNWVERNSYSCSVVHEGLHNHHTTKSFSRTPGK

SEQ ID NO: 35 - DNA, 648 bp, synthetic construct
  source 1..648: mol_type = other DNA; note = tA3-20.3_mouse_LC
aattttatgctgactcagccccactctgtgtcggagtctccggggaagacggtaaacatctcctgcacccgcagcagtggcagcattgccaccaactatgtgcagtggtaccagcagcgccccggcagttcccccaccactgtgatctatgaggataaccaaagaccctctggggtccctgatcggttctctggctccatcgacagctcctccaactctgcctccctcaccatctctggactgaagactgaggacgaggctgtctatcactgtcagtcttatgatagcagcaatgtggtattcggcggagggaccaagctgaccgtcctaggccagcctaagtcctctccttccgtgactctgttccctccatcctccgaggaactggaaacaaacaaggctaccctcgtgtgcaccatcaccgacttctatcctggcgtggtcaccgtggactggaaggtggacggaacccctgtgacacaaggcatggaaaccacacagccctccaagcagtccaacaacaagtacatggcctccagctatctgaccctgaccgctagagcttgggagagacactcctcctacagctgccaagtgacccacgagggccacaccgtggaaaagtctctgtctagagccgactgctcc

SEQ ID NO: 36 - protein, 216 aa, synthetic construct
  source 1..216: note = tA3-20.3_mouse_LC
NFMLTQPHSVSESPGKTVNISCTRSSGSIATNYVQWYQQRPGSSPTTVIYEDNQRPSGVPDRFSGSIDSSSNSASLTISGLKTEDEAVYHCQSYDSSNVVFGGGTKLTVLGQPKSSPSVTLFPPSSEELETNKATLVCTITDFYPGVVTVDWKVDGTPVTQGMETTQPSKQSNNKYMASSYLTLTARAWERHSSYSCQVTHEGHTVEKSLSRADCS

SEQ ID NO: 37 - DNA, 1434 bp, synthetic construct
  source 1..1434: mol_type = other DNA; note = 371M_scFv_mouse Fc
gaagtgcagctggttgaatctggcggcggagttgttcagcctggcggatctctgagactgtcttgtgccgcctccggcttcaccttctcctcttacgctatgtcctgggtccgacaggcccctggcaaatgtctggaatgggtgtccgccatctctggctctggcggctctacctactacgccgactctgtgaagggcagattcaccatcagccgggacaactccaagaacaccctgtacctgcagatgaactccctgagagccgaggacaccgccgtgtactactgtgctaagggcacccgcaccaactggtacttcgatctgtggggcagaggcaccctggtcacagtttctagcggaggcggaggatcaggtggcggtggatctggcggtggcggatcctcttatgagctgacccaacctccttccgcctctggcacacctggacagagagtgaccatctcctgctccggctctcggtccaacatcggctctaacaccgtgaactggtatcagcaggtccccggcacagctcccaagctgctgatctactccaacaaccagcggccttctggcgtgcccgatagattcagcggctctaagtctggcacctctgccagcctggctatcagtggactgcagagcgaggatgaggctgagtactactgcgccgcctgggacgattctctgtacggccctgtgtttggctgtggcacccagctgacagtgctgggagaacctaggggccctaccatcaagccttgtcctccatgcaagtgccccgctcctaatgctgctggtggcccttccgtgttcatcttcccacctaagatcaaggacgtgctgatgatctccctgtctcctatcgtgacctgcgtggtggtggacgtgtccgaggatgatcctgacgtgcagatcagttggttcgtgaacaacgtggaagtgcacaccgctcagacccagacacacagagaggactacaacagcaccctgagagtggtgtctgccctgcctatccagcaccaggattggatgtccggcaaagagttcaagtgcaaagtgaacaacaaggacctggccgctcctatcgagcggaccatctctaagcctaagggctctgtcagggccccacaggtgtacgttttgcctccacctgaggaagagatgaccaagaaacaggtgtccctgacctgcctggtcaaggacttcatgcccgaggacatctacgtggaatggaccaacaacggcaagaccgagctgaattacaagaacacagagcccgtgctggactccgacggctcctacttcatgtactccgagctgaccgtcgagaagaagaactgggtcgagagaaactcctactcctgcagcgtggtgcacgagggcctgcacaatcaccacaccaccgacagcttcagcagaaccccaggcaag

SEQ ID NO: 38 - protein, 478 aa, synthetic construct
  source 1..478: note = 371M_scFv_mouse Fc
EVQLVESGGGVVQPGGSLRLSCAASGFTFSSYAMSWVRQAPGKCLEWVSAISGSGGSTYYADSVKGRFTISRDNSKNTLYLQMNSLRAEDTAVYYCAKGTRTNWYFDLWGRGTLVTVSSGGGGSGGGGSGGGGSSYELTQPPSASGTPGQRVTISCSGSRSNIGSNTVNWYQQVPGTAPKLLIYSNNQRPSGVPDRFSGSKSGTSASLAISGLQSEDEAEYYCAAWDDSLYGPVFGCGTQLTVLGEPRGPTIKPCPPCKCPAPNAAGGPSVFIFPPKIKDVLMISLSPIVTCVVVDVSEDDPDVQISWFVNNVEVHTAQTQTHREDYNSTLRVVSALPIQHQDWMSGKEFKCKVNNKDLAAPIERTISKPKGSVRAPQVYVLPPPEEEMTKKQVSLTCLVKDFMPEDIYVEWTNNGKTELNYKNTEPVLDSDGSYFMYSELTVEKKNWVERNSYSCSVVHEGLHNHHTTDSFSRTPGK

SEQ ID NO: 39 - protein, 217 aa, synthetic construct
  source 1..217: note = tA3-20_Fc
APEAAGGPSVFLFPPKPKDTLMISRTPEVTCVVVDVSHEDPEVKFNWYVDGVEVHNAKTKPREEQYNSTYRVVSVLTVLHQDWLNGKEYKCKVSNKALPAGIEKTISKAKGQPREPQVYTLPPSRDELTKNQVSLTCLVKGFYPSDIAVEWESNGQPENNYKTTPPVLDSDGSFFLYSKLTVDKSRWQQGNVFSCSVMHEALHNHYTQKSLSLSPGK

SEQ ID NO: 40 - protein, 217 aa, synthetic construct
  source 1..217: note = tA3-20_human 371M_Fc_knob
APEAAGGPSVFLFPPKPKDTLMISRTPEVTCVVVDVSHEDPEVKFNWYVDGVEVHNAKTKPREEQYNSTYRVVSVLTVLHQDWLNGKEYKCKVSNKALPAGIEKTISKAKGQPREPQVYTLPPSRDELTKNQVSLWCLVKGFYPSDIAVEWESNGQPENNYKTTPPVLDSDGSFFLYSKLTVDKSRWQQGNVFSCSVMHEALHNHYTQKSLSLSPGK

SEQ ID NO: 41 - protein, 217 aa, synthetic construct
  source 1..217: note = tA3-20_human 371M_Fc_hole
APEAAGGPSVFLFPPKPKDTLMISRTPEVTCVVVDVSHEDPEVKFNWYVDGVEVHNAKTKPREEQYNSTYRVVSVLTVLHQDWLNGKEYKCKVSNKALPAGIEKTISKAKGQPREPQVYTLPPSRDELTKNQVSLSCAVKGFYPSDIAVEWESNGQPENNYKTTPPVLDSDGSFFLVSKLTVDKSRWQQGNVFSCSVMHEALHNHYTQKSLSLSPGK

SEQ ID NO: 42 - protein, 15 aa, synthetic construct
  source 1..15: note = Hinge
EPKSCDKTHTCPPCP

SEQ ID NO: 43 - protein, 245 aa, synthetic construct
  source 1..245: note = 371M_scFv
EVQLVESGGGVVQPGGSLRLSCAASGFTFSSYAMSWVRQAPGKCLEWVSAISGSGGSTYYADSVKGRFTISRDNSKNTLYLQMNSLRAEDTAVYYCAKGTRTNWYFDLWGRGTLVTVSSGGGGSGGGGSGGGGSSYELTQPPSASGTPGQRVTISCSGSRSNIGSNTVNWYQQVPGTAPKLLIYSNNQRPSGVPDRFSGSKSGTSASLAISGLQSEDEAEYYCAAWDDSLYGPVFGCGTQLTVLG

SEQ ID NO: 44 - protein, 449 aa, synthetic construct
  source 1..449: note = 371M_HC_control
EVQLVESGGGVVQPGGSLRLSCAASGFTFSSYAMSWVRQAPGKGLEWVSAISGSGGSTYYADSVKGRFTISRDNSKNTLYLQMNSLRAEDTAVYYCAKGTRTNWYFDLWGRGTLVTVSSAKTTAPSVYPLAPVCGDTTGSSVTLGCLVKGYFPEPVTLTWNSGSLSSGVHTFPAVLQSDLYTLSSSVTVTSSTWPSQSITCNVAHPASSTKVDKKIEPRGPTIKPCPPCKCPAPNLLGGPSVFIFPPKIKDVLMISLSPIVTCVVVDVSEDDPDVQISWFVNNVEVHTAQTQTHREDYNSTLRVVSALPIQHQDWMSGKEFKCKVNNKDLPAPIERTISKPKGSVRAPQVYVLPPPEEEMTKKQVTLTCMVTDFMPEDIYVEWTNNGKTELNYKNTEPVLDSDGSYFMYSKLRVEKKNWVERNSYSCSVVHEGLHNHHTTKSFSRTPGK

SEQ ID NO: 45 - protein, 216 aa, synthetic construct
  source 1..216: note = 371M_LC_control
SYELTQPPSASGTPGQRVTISCSGSRSNIGSNTVNWYQQVPGTAPKLLIYSNNQRPSGVPDRFSGSKSGTSASLAISGLQSEDEAEYYCAAWDDSLYGPVFGGGTQLTVLGQPKSSPSVTLFPPSSEELETNKATLVCTITDFYPGVVTVDWKVDGTPVTQGMETTQPSKQSNNKYMASSYLTLTARAWERHSSYSCQVTHEGHTVEKSLSRADCS

SEQ ID NO: 46 - protein, 4 aa, synthetic construct
  source 1..4: note = GS_linker_1
GGGS

SEQ ID NO: 47 - protein, 4 aa, synthetic construct
  source 1..4: note = GS_linker_2
SGGG

SEQ ID NO: 48 - protein, 5 aa, synthetic construct
  source 1..5: note = GS_linker_3
GGGGS

SEQ ID NO: 49 - protein, 5 aa, synthetic construct
  source 1..5: note = GS_linker_4
SGGGG

SEQ ID NO: 50 - protein, 6 aa, synthetic construct
  source 1..6: note = GS_linker_5
GGGGGS

SEQ ID NO: 51 - protein, 6 aa, synthetic construct
  source 1..6: note = GS_linker_6
SGGGGG

SEQ ID NO: 52 - protein, 7 aa, synthetic construct
  source 1..7: note = GS_linker_7
GGGGGGS

SEQ ID NO: 53 - protein, 7 aa, synthetic construct
  source 1..7: note = GS_linker_8
SGGGGGG

SEQ ID NO: 54 - protein, 15 aa, synthetic construct
  source 1..15: note = GS_linker_9
GGGGSGGGGSGGGGS

SEQ ID NO: 55 - protein, 5 aa, synthetic construct
  source 1..5: note = GS_linker_10
GKPGS

SEQ ID NO: 56 - DNA, 1359 bp, synthetic construct
  source 1..1359: mol_type = other DNA; note = 2A4-VH_CK_Fc_knob
gaggttcaacttgttgaaagtggcggaagattagtgcagcccaaaggctccctcaaactgtcttgtgctgcaagtggctttacgtttaacacctatgccatgtattggatccggcaggcaccaggtaaagggttagaatgggtggcacgaatccgcagtaagtcaaataactacgccatctactacgccgacagcgttaaagataggttcaccatcttccgcgacgacagccagagcatgctgtatctccagatgaacaacctgaagacggaggataccgctatgtactactgcgtcaggccctactcagacagtttcgcctattggggccagggtactcttgtaactgtctcctccgctagcgtggcggccccatctgtatttattttccctccatcagatgagcagcttaagtcaggaaccgcttccgtggtgtgcctgctaaacaacttctatccccgggaggcaaaggtccaatggaaagtagacaatgccctccagagcgggaactctcaagaatctgtgacagagcaagatagtaaggattcgacctactccctgagctccacacttacactcagcaaagcagactacgagaagcacaaagtctacgcctgcgaggttacacaccagggcctgagtagccctgtcacaaaatcatttaaccggggcgaatgcgacaagactcacacatgtcctccatgtcctgctccagaagctgctggtggaccatctgtatttctctttcctcccaagcccaaggacacacttatgatttcacgaacacccgaagtgacctgtgtggtggtcgatgtgtcccatgaggatcctgaggtcaaattcaactggtacgtggacggcgtggaggttcataatgctaaaactaagcccagggaggagcagtataatagcacttatcgcgtggtctcggtgctcactgttttgcatcaggactggctgaacgggaaagaatataagtgtaaggtgagcaataaggccctgcctgctggaatagagaagacaattagcaaggccaaggggcagccaagagaacctcaagtatataccctcccgccctctagagatgaattgactaagaatcaggtgagcctgtggtgcctggtgaaaggattttatcccagcgacatcgctgtggagtgggaaagtaacggccagcctgaaaataactacaagaccactccgcccgtgctggattctgatggttctttctttctgtactccaagctgaccgtggacaagtctcgttggcagcagggcaatgtcttctcatgctctgtgatgcacgaggcactacacaatcactacacccagaagtccctgtccttgtctccaggaaaa

SEQ ID NO: 57 - protein, 453 aa, synthetic construct
  source 1..453: note = 2A4-VH_CK_Fc_knob
EVQLVESGGRLVQPKGSLKLSCAASGFTFNTYAMYWIRQAPGKGLEWVARIRSKSNNYAIYYADSVKDRFTIFRDDSQSMLYLQMNNLKTEDTAMYYCVRPYSDSFAYWGQGTLVTVSSASVAAPSVFIFPPSDEQLKSGTASVVCLLNNFYPREAKVQWKVDNALQSGNSQESVTEQDSKDSTYSLSSTLTLSKADYEKHKVYACEVTHQGLSSPVTKSFNRGECDKTHTCPPCPAPEAAGGPSVFLFPPKPKDTLMISRTPEVTCVVVDVSHEDPEVKFNWYVDGVEVHNAKTKPREEQYNSTYRVVSVLTVLHQDWLNGKEYKCKVSNKALPAGIEKTISKAKGQPREPQVYTLPPSRDELTKNQVSLWCLVKGFYPSDIAVEWESNGQPENNYKTTPPVLDSDGSFFLYSKLTVDKSRWQQGNVFSCSVMHEALHNHYTQKSLSLSPGK

SEQ ID NO: 58 - DNA, 651 bp, synthetic construct
  source 1..651: mol_type = other DNA; note = 2A4-VK_CH1
gacgttgttatgacacaaactccactctctttaccagtctctctaggggatcaggccagcattagctgccgatcttctcagagtctggtccattcaaccggaaatacctatctgcactggtacctccagaagcccggtcaatctccaaaactgctgatctacaaggtcagcaaccgcttcagcggcgtaccagatagattttccggctccggcagcggcacatacttcacactcaaaattagcagggtcgaggcagaagatcttggtgtgtatttctgcagccagtccacccacgtccctttcacttttggaggtggaacgaagctcgagatcaagagctccgctagcacaaaaggcccttcagtatttcctctggcccctagtagcaagtccacaagtggcggcacagcagctctgggatgtctcgttaaagactatttccccgaacccgtcaccgtgtcctggaactctggggctctgacttctggagttcatacctttcccgctgtgttgcagtcgtccgggctgtacagtctgtcttcagtggtgactgtgcccagttcttcactggggactcagacatacatctgcaacgtgaaccacaagccctcaaataccaaggtggacaagaaggtggagccgaaaagttgt

SEQ ID NO: 59 - protein, 217 aa, synthetic construct
  source 1..217: note = 2A4-VK_CH1
DVVMTQTPLSLPVSLGDQASISCRSSQSLVHSTGNTYLHWYLQKPGQSPKLLIYKVSNRFSGVPDRFSGSGSGTYFTLKISRVEAEDLGVYFCSQSTHVPFTFGGGTKLEIKSSASTKGPSVFPLAPSSKSTSGGTAALGCLVKDYFPEPVTVSWNSGALTSGVHTFPAVLQSSGLYSLSSVVTVPSSSLGTQTYICNVNHKPSNTKVDKKVEPKSC

SEQ ID NO: 60 - DNA, 1347 bp, synthetic construct
  source 1..1347: mol_type = other DNA; note = tA3-20_HC_hole
caggtgcagctggttcagtctggcgccgaagtgaagaaacctggctcctccgtgaaggtgtcctgcaaggcttctggcggcaccttcaactcctacgccatctcttggatgagacaggcccctggacagggccttgaatggatgggaggcatcatccccatcttcggccctgctaagcacgcccagaaattccagggcagagtgaccatcaccgccgacaagtctacctccaccgtgtacatggaactgtccagcctgagatccgaggacaccgccgtgtactactgtgctagactcgtgggcgctaccggatggttcgatccttggggacagggcacactggtcaccgtgtcctctgcttctaccaagggacccagcgtgttccctctggctcctagctctaagtccacctccggtggaacagctgctctgggctgtctggtcaaggactacttccctgagcctgtgaccgtgtcttggaactctggcgctctgacatccggcgtgcacacctttccagctgtgctgcaatcctccggcctgtactctctgtcctccgtcgtgaccgtgccttctagctctctgggcacccagacctacatctgcaatgtgaaccacaagccttccaacaccaaggtggacaagaaggtggaacccaagtcctgcgacaagacccacacctgtcctccatgtcctgctccagaagctgcaggcggcccttccgtgtttctgttccctccaaagcctaaggacaccctgatgatctctcggacccctgaagtgacctgcgtggtggtggatgtgtctcacgaggacccagaagtgaagttcaattggtacgtggacggcgtggaagtgcacaacgccaagaccaagcctagagaggaacagtacaactccacctacagagtggtgtccgtgctgaccgtgctgcaccaggattggctgaacggcaaagagtacaagtgcaaggtgtccaacaaggcactgcctgccggcatcgaaaagaccatctccaaggctaagggccagcctcgggaaccccaggtttacacattgcctccatctcgggacgagctgaccaagaaccaggtgtccctgtcttgtgccgtgaagggcttctacccctccgatatcgctgtggaatgggagtccaatggccagccagagaacaactacaagacaacccctcctgtgctggactccgacggctcattcttcctggtgtccaagctgacagtggacaagtccagatggcagcagggcaacgtgttctcctgctccgtgatgcacgaggccctgcacaatcactacacacagaagtctctgtctctgtcccctggcaag

SEQ ID NO: 61 - protein, 449 aa, synthetic construct
  source 1..449: note = tA3-20_HC_hole
QVQLVQSGAEVKKPGSSVKVSCKASGGTFNSYAISWMRQAPGQGLEWMGGIIPIFGPAKHAQKFQGRVTITADKSTSTVYMELSSLRSEDTAVYYCARLVGATGWFDPWGQGTLVTVSSASTKGPSVFPLAPSSKSTSGGTAALGCLVKDYFPEPVTVSWNSGALTSGVHTFPAVLQSSGLYSLSSVVTVPSSSLGTQTYICNVNHKPSNTKVDKKVEPKSCDKTHTCPPCPAPEAAGGPSVFLFPPKPKDTLMISRTPEVTCVVVDVSHEDPEVKFNWYVDGVEVHNAKTKPREEQYNSTYRVVSVLTVLHQDWLNGKEYKCKVSNKALPAGIEKTISKAKGQPREPQVYTLPPSRDELTKNQVSLSCAVKGFYPSDIAVEWESNGQPENNYKTTPPVLDSDGSFFLVSKLTVDKSRWQQGNVFSCSVMHEALHNHYTQKSLSLSPGK

SEQ ID NO: 62 - DNA, 1347 bp, synthetic construct
  source 1..1347: mol_type = other DNA; note = 2A4_HC_control
gaggttcaacttgttgaaagtggcggaagattagtgcagcccaaaggctccctcaaactgtcttgtgctgcaagtggctttacgtttaacacctatgccatgtattggatccggcaggcaccaggtaaagggttagaatgggtggcacgaatccgcagtaagtcaaataactacgccatctactacgccgacagcgttaaagataggttcaccatcttccgcgacgacagccagagcatgctgtatctccagatgaacaacctgaagacggaggataccgctatgtactactgcgtcaggccctactcagacagtttcgcctattggggccagggtactcttgtaactgtctccgctgctagcaccaagggacccagcgtgttccctctggctcctagctctaagtccacctctggcggaacagctgctctgggctgtctggtcaaggactacttccctgagcctgtgaccgtgtcctggaactctggcgctctgacatctggcgtgcacacattccctgctgtgctgcagtcctccggcctgtactctctgtcctctgtcgtgaccgtgccttccagctctctgggaacccagacctacatctgcaatgtgaaccacaagccttccaacaccaaggtggacaagaaggtggaacccaagtcctgcgacaagacccacacctgtcctccatgtcctgctccagaactgctcggcggaccttccgtgttcctgtttcctccaaagcctaaggacaccctgatgatctctcggacccctgaagtgacctgcgtggtggtggatgtgtctcacgaggacccagaagtgaagttcaattggtacgtggacggcgtggaagtgcacaacgccaagaccaagcctagagaggaacagtacaactccacctacagagtggtgtccgtgctgaccgtgctgcaccaggattggctgaacggcaaagagtacaagtgcaaggtgtccaacaaggccctgcctgctcctatcgaaaagaccatctccaaggccaagggccagcctagggaaccccaggtttacaccttgcctccatctcgggacgagctgaccaagaaccaggtgtccctgacctgtctcgtgaagggcttctacccttccgatatcgccgtggaatgggagtctaacggccagccagagaacaactacaagacaacccctcctgtgctggactccgacggctcattcttcctgtactccaagctgacagtggataagtcccggtggcagcagggcaacgtgttctcttgctctgtgatgcacgaggccctgcacaaccactacacacagaagtctctgtctctgagccccggcaag

SEQ ID NO: 63 - protein, 449 aa, synthetic construct
  source 1..449: note = 2A4_HC_control
EVQLVESGGRLVQPKGSLKLSCAASGFTFNTYAMYWIRQAPGKGLEWVARIRSKSNNYAIYYADSVKDRFTIFRDDSQSMLYLQMNNLKTEDTAMYYCVRPYSDSFAYWGQGTLVTVSAASTKGPSVFPLAPSSKSTSGGTAALGCLVKDYFPEPVTVSWNSGALTSGVHTFPAVLQSSGLYSLSSVVTVPSSSLGTQTYICNVNHKPSNTKVDKKVEPKSCDKTHTCPPCPAPELLGGPSVFLFPPKPKDTLMISRTPEVTCVVVDVSHEDPEVKFNWYVDGVEVHNAKTKPREEQYNSTYRVVSVLTVLHQDWLNGKEYKCKVSNKALPAPIEKTISKAKGQPREPQVYTLPPSRDELTKNQVSLTCLVKGFYPSDIAVEWESNGQPENNYKTTPPVLDSDGSFFLYSKLTVDKSRWQQGNVFSCSVMHEALHNHYTQKSLSLSPGK

SEQ ID NO: 64 - DNA, 657 bp, synthetic construct
  source 1..657: mol_type = other DNA; note = 2A4_LC_control
gacgttgttatgacacaaactccactctctttaccagtctctctaggggatcaggccagcattagctgccgatcttctcagagtctggtccattcaaccggaaatacctatctgcactggtacctccagaagcccggtcaatctccaaaactgctgatctacaaggtcagcaaccgcttcagcggcgtaccagatagattttccggctccggcagcggcacatacttcacactcaaaattagcagggtcgaggcagaagatcttggtgtgtatttctgcagccagtccacccacgtccctttcacttttggaggtggaacgaagctcgagatcaagcgtacggtggccgctccttccgtgttcatcttcccaccttccgacgagcagctgaagtccggcacagcttctgtcgtgtgcctgctgaacaacttctaccctcgggaagccaaggtgcagtggaaggtggacaatgccctgcagtccggcaactcccaagagtctgtgaccgagcaggactccaaggacagcacctacagcctgtcctccacactgaccctgtccaaggccgactacgagaagcacaaggtgtacgcctgcgaagtgacccatcagggcctgtctagccctgtgaccaagtctttcaaccggggcgagtgc

SEQ ID NO: 65 - protein, 219 aa, synthetic construct
  source 1..219: note = 2A4_LC_control
DVVMTQTPLSLPVSLGDQASISCRSSQSLVHSTGNTYLHWYLQKPGQSPKLLIYKVSNRFSGVPDRFSGSGSGTYFTLKISRVEAEDLGVYFCSQSTHVPFTFGGGTKLEIKRTVAAPSVFIFPPSDEQLKSGTASVVCLLNNFYPREAKVQWKVDNALQSGNSQESVTEQDSKDSTYSLSSTLTLSKADYEKHKVYACEVTHQGLSSPVTKSFNRGEC

SEQ ID NO: 66 - DNA, 1350 bp, synthetic construct
  source 1..1350: mol_type = other DNA; note = M6_HC_control
caagtgaagctggaagagtctggccccgagctgaagaaacctggcgagacagtgaagatctcctgcaaggcctccggctacaccttcaccaactacggcatgaactgggtcaagcaggctcctggcaagggcctgaaatggatgggctggatcaacacctacaccggcgagcctacctacgccgacgatttcaagggcagattcgtgttctccctggaaacctccgcctccaccgcttacctgcagatcaacaacctgaagaacgaggacatggccacctacttttgcgcccggaagtccaccgtggtgtccagatacttcgatgtgtggggcgctggcaccaccgtgacagtgtcctctgctagcacaaagggcccctctgtgttccctctggctcctagctctaagtccacctctggcggaacagctgctctgggctgtctggtcaaggactacttccctgagcctgtgaccgtgtcttggaactctggcgctctgacatccggcgtgcacacatttccagctgtgctgcagtcctccggcctgtactctctgtcctctgtcgtgaccgtgccttccagctctctgggaacccagacctacatctgcaatgtgaaccacaagccttccaacaccaaggtggacaagaaggtggaacccaagtcctgcgacaagacccacacctgtcctccatgtcctgctccagaagctgctggcggaccttccgtgttcctgtttcctccaaagcctaaggacaccctgatgatctctcggacccctgaagtgacctgcgtggtggtggatgtgtctcacgaggacccagaagtgaagttcaattggtacgtggacggcgtggaagtgcacaacgccaagaccaagcctagagaggaacagtacaactccacctacagagtggtgtccgtgctgaccgtgctgcaccaggattggctgaacggcaaagagtacaagtgcaaggtgtccaacaaggccctgcctgccggcatcgaaaagaccatctccaaggccaagggccagcctagggaaccccaggtttacaccttgccaccttctcgggacgagctgaccaagaaccaggtgtccctgacctgtctcgtgaagggcttctacccctccgatatcgccgtggaatgggagtctaatggccagcctgagaacaactacaagacaacccctcctgtgctggactccgacggctcattcttcctgtactccaagctgacagtggacaagtccagatggcagcagggcaacgtgttctcctgcagcgtgatgcacgaggccctgcacaatcactacacacagaagtctctgtctctgagccccggcaag

SEQ ID NO: 67 - protein, 450 aa, synthetic construct
  source 1..450: note = M6_HC_control
QVKLEESGPELKKPGETVKISCKASGYTFTNYGMNWVKQAPGKGLKWMGWINTYTGEPTYADDFKGRFVFSLETSASTAYLQINNLKNEDMATYFCARKSTVVSRYFDVWGAGTTVTVSSASTKGPSVFPLAPSSKSTSGGTAALGCLVKDYFPEPVTVSWNSGALTSGVHTFPAVLQSSGLYSLSSVVTVPSSSLGTQTYICNVNHKPSNTKVDKKVEPKSCDKTHTCPPCPAPEAAGGPSVFLFPPKPKDTLMISRTPEVTCVVVDVSHEDPEVKFNWYVDGVEVHNAKTKPREEQYNSTYRVVSVLTVLHQDWLNGKEYKCKVSNKALPAGIEKTISKAKGQPREPQVYTLPPSRDELTKNQVSLTCLVKGFYPSDIAVEWESNGQPENNYKTTPPVLDSDGSFFLYSKLTVDKSRWQQGNVFSCSVMHEALHNHYTQKSLSLSPGK

SEQ ID NO: 68 - DNA, 642 bp, synthetic construct
  source 1..642: mol_type = other DNA; note = M6_LC_control
gacatcgtgctgacccagacacacaagttcatgtccacctccgtgggcgacagagtgtccatcacatgcaaggcctctcaggatgtgggcgacgctgtgacatggtgccagcagaaacctggccagcctcctaagctgctgatctactgggcctctaccagacataccggcgtgcccgatagattcaccggctctggctctggcaccgacttcaccctgaccatcaacaacgtgcagtccgaggacctggccgactacttctgccagcagtaccggtcttaccctctgacctttggagccggcaccaagctggaactgaagcgtacggtggccgctccttccgtgttcatcttcccaccttccgacgagcagctgaagtccggcacagcttctgtcgtgtgcctgctgaacaacttctaccctcgggaagccaaggtgcagtggaaggtggacaatgccctgcagtccggcaactcccaagagtctgtgaccgagcaggactccaaggacagcacctacagcctgtcctccacactgaccctgtccaaggccgactacgagaagcacaaggtgtacgcctgcgaagtgacccatcagggcctgtctagccctgtgaccaagtctttcaaccggggcgagtgc

SEQ ID NO: 69 - protein, 214 aa, synthetic construct
  source 1..214: note = M6_LC_control
DIVLTQTHKFMSTSVGDRVSITCKASQDVGDAVTWCQQKPGQPPKLLIYWASTRHTGVPDRFTGSGSGTDFTLTINNVQSEDLADYFCQQYRSYPLTFGAGTKLELKRTVAAPSVFIFPPSDEQLKSGTASVVCLLNNFYPREAKVQWKVDNALQSGNSQESVTEQDSKDSTYSLSSTLTLSKADYEKHKVYACEVTHQGLSSPVTKSFNRGEC

SEQ ID NO: 70 - protein, 15 aa, synthetic construct
  source 1..15: note = Hinge2
EPKSSDKTHTCPPCP